European Patent Application EP 4 311 553 A1, published January 31, 2024. Title: Preparation Method of Gynostemma pentaphyllum Leaves Extract and Gynostemma pentaphyllum Leaves Extract Using The Same. Applicant: Bionic Trading Corporation). Application EP 23178063.6, filed June 7, 2023. The sequence listing filed with the application follows.

SEQUENCE LISTING (18 sequences)

SEQ ID NO: 1 - DNA, 20 bp, synthetic construct
  source 1..20: mol_type = other DNA
gtccagagagtcggcaagtc

SEQ ID NO: 2 - DNA, 20 bp, synthetic construct
  source 1..20: mol_type = other DNA
gtcggtgatcgtgagacctt

SEQ ID NO: 3 - DNA, 20 bp, synthetic construct
  source 1..20: mol_type = other DNA
tctactcggccacaggcgct

SEQ ID NO: 4 - DNA, 20 bp, synthetic construct
  source 1..20: mol_type = other DNA
cttgacagctcccgccgcaa

SEQ ID NO: 5 - DNA, 22 bp, synthetic construct
  source 1..22: mol_type = other DNA
ctgtgtggattggtggctctat

SEQ ID NO: 6 - DNA, 23 bp, synthetic construct
  source 1..23: mol_type = other DNA
gtgtaaaacgcagctcagtaaca

SEQ ID NO: 7 - DNA, 20 bp, synthetic construct
  source 1..20: mol_type = other DNA
ggatggtgcccctgggtcct

SEQ ID NO: 8 - DNA, 20 bp, synthetic construct
  source 1..20: mol_type = other DNA
tggccttcgctgtgagtcgc

SEQ ID NO: 9 - DNA, 20 bp, synthetic construct
  source 1..20: mol_type = other DNA
tgggctgccacaagccagac

SEQ ID NO: 10 - DNA, 20 bp, synthetic construct
  source 1..20: mol_type = other DNA
cagcccagccactggcatca

SEQ ID NO: 11 - DNA, 20 bp, synthetic construct
  source 1..20: mol_type = other DNA
atgtgtcgccttcttgctct

SEQ ID NO: 12 - DNA, 20 bp, synthetic construct
  source 1..20: mol_type = other DNA
atctactgcctggggacctt

SEQ ID NO: 13 - DNA, 20 bp, synthetic construct
  source 1..20: mol_type = other DNA
aaggggatggagaccacagt

SEQ ID NO: 14 - DNA, 20 bp, synthetic construct
  source 1..20: mol_type = other DNA
tgaggtgggagctgataggg

SEQ ID NO: 15 - DNA, 20 bp, synthetic construct
  source 1..20: mol_type = other DNA
tggacccaagcattacggac

SEQ ID NO: 16 - DNA, 20 bp, synthetic construct
  source 1..20: mol_type = other DNA
ggtcatttcaccgccctgta

SEQ ID NO: 17 - DNA, 20 bp, synthetic construct
  source 1..20: mol_type = other DNA
gcttccaggaggctaaggat

SEQ ID NO: 18 - DNA, 20 bp, synthetic construct
  source 1..20: mol_type = other DNA
cccaatcccaatgacaactc